European Patent Specification EP 3 526 236 B1, published December 10, 2025. Title: SIGNATURE-BASED HUMAN IMMUNODEFICIENCY VIRUS (HIV) ENVELOPE (ENV) TRIMER VACCINES AND METHODS OF USING THE SAME. Applicant: Beth Israel Deaconess Medical Center, Inc. Los Alamos National Security, LLC. The sequence listing filed with the application follows.

SEQUENCE LISTING (46 sequences)

SEQ ID NO: 1 - protein, 645 aa, Artificial Sequence
  Synthetic construct
VGNLWVTVYYGVPVWREAKTTLFCASDAKAYDREVHNVWATHACVPTDPNPQEIVLENVTENFNMWKNDMVDQMHEDIISLWDQSLKPCVKLTPLCVTLECTAFNSSSHTNSSIAMQEMKNCSFNMTTELRDKKKKVSALFYKLDIVPLNKNGRQYRLINCNTSTLTQACPKVSFDPIPIHYCTPAGYAILKCNNKTFNGTGPCNNVSTVQCTHGIKPVVSTQLLLNGSLAEEDIIIRSENLTNNAKTIIVHLNESVEIVCIRPNNNTRKSIRIGPGQTFYANNDIIGDIRQAHCNISKEKWNNTLHRVWKKLVEHFPNKTTIRFDRHSGGDLEITTHSFNCGGEFFYCNTSGLFNITYNSNYTYNDTKHNGTKVITLPCRIKQIINMWQEVGRAMYAPPIAGNITCTSNITGLLLTRDGGNNSTETETFRPGGGDMRDNWRSELYKYKVVEIKPLGIAPTGAKRRVVEREKRAVGIGAVFLGFLGAAGSTMGAASITLTVQARQLLSGIVQQQSNLLKAIEAQQHLLQLTVWGIKQLQTRVLAIERYLKDQQLLGLWGCSAKLICTTAVPWNSSWSNKSETEIWNNMTWMQWDREISNYTNTIYRLLEESQNQQEKNENDLLALDKWNSLWDWFGISNWLWYIR

SEQ ID NO: 2 - protein, 645 aa, Artificial Sequence
  Synthetic construct
VGNLWVTVYYGVPVWREAETTLFCASDAKAYDREVHNVWATHACVPTDPNPQEIVLENVTENFNMWKNDMVDQMHEDIISLWDQSLKPCVKLTPLCVTLDCKAFNSSSHTNSSIAMQEMKNCTFNITTSVKGKRQQEHALFYKLDIVPLNKNGRQYRLINCNTSTLTQACPKVSFDPIPIHYCTPAGYAILKCNNKTFNGTGPCNNVSTVQCTHGIKPVVSTQLLLNGSLAEEDIIIRSENLTNNAKTIIVHLNESVEIVCVRPNNNTRKSIRIGPGQTFYANNEIIGDIRQAHCNISKEKWNNTLHRVWKKLVEHFPNKTTIRFDRHSGGDLEITTHSFNCGGEFFYCNTSGLFNITYNSNYTYNDTKHNGTKVITLPCRIKQIINMWQEVGRAMYAPPIAGNITCTSNITGLLLTRDGGNNSTETETFRPGGGDMRDNWRSELYKYKVVEIKPLGIAPTGAKRRVVEREKRAVGIGAVFLGFLGAAGSTMGAASITLTVQARQLLSGIVQQQSNLLKAIEAQQHLLQLTVWGIKQLQTRVLAIERYLKDQQLLGLWGCSAKLICTTAVPWNSSWSNKSETEIWNNMTWMQWDREISNYTNTIYRLLEESQNQQEKNENDLLALDKWNSLWDWFGISNWLWYIR

SEQ ID NO: 3 - protein, 645 aa, Artificial Sequence
  Synthetic construct
VGNLWVTVYYGVPVWREAKTTLFCASDAKAYDREVHNVWATHACVPTDPNPQEIVLENVTENFNMWKNDMVDQMHEDIISLWDQSLKPCVKLTPLCVTLNCTAFNSSSHTNSSIAMQEMKNCSFKATTEIRDRKKEMYALFYKLDIVPINKNGRQYRLINCNTSTLTQACPKVSFDPIPIHYCTPAGFAILKCNNKTFNGTGPCTNVSTVQCTHGIKPVVSTQLLLNGSLAEEDIIIRSENLTNNAKTIIVHLNESVEINCTRPGNNTRKSIRIGPGQTFYANNDIIGDIRQAHCNISEAKWNNTLHQVAKKLVEHFPNKTTIRFDRHSGGDLEITTHSFNCGGEFFYCNTSGLFNITYNSNYTYNDTKHNGTKVITLPCRIKQIINMWQEVGRAMYAPPIAGNITCTSNITGLLLTRDGGNNSTETETFRPGGGDMRDNWRSELYKYKVVEIKPLGIAPTGAKRRVVEREKRAVGIGAVFLGFLGAAGSTMGAASITLTVQARQLLSGIVQQQSNLLKAIEAQQHLLQLTVWGIKQLQTRVLAIERYLKDQQLLGLWGCSAKLICTTAVPWNSSWSNKSETEIWNNMTWMQWDREINNYTNTIYRLLEESQNQQEKNENDLLALDKWNSLWDWFGISNWLWYIR

SEQ ID NO: 4 - protein, 645 aa, Artificial Sequence
  Synthetic construct
VGNLWVTVYYGVPVWREAKTTLFCASDAKAYDREVHNVWATHACVPTDPNPQEIVLENVTENFNMWKNDMVDQMHEDIISLWDQSLKPCVKLTPLCVTLNCTAFNSSSHTNSSIAMQEMKNCSFNATTEIRDRKKEMYALFYKLDIVPINKNGRQYRLINCNTSTLTQACPKVSFDPIPIHYCTPAGFAILKCNNKTFNGTGPCTNVSTVQCTHGIKPVVSTQLLLNGSLAEEDIIIRSENLSNNAKTIIVHLNESVEITCIRPSNNTRKSVRIGPGQTFYANNDIIGNIRKAYCEINETKWNNTLHNVSKKLVEHFPNKTTIRFDRHSGGDLEITTHSFNCGGEFFYCNTSGLFNISYNSNYTYNDTKHNGTKVITLPCRIKQIINMWQEVGRAMYAPPIAGNITCTSNITGLLLTRDGGNNSTETETFRPGGGDMRDNWRSELYKYKVVEIKPLGIAPTGAKRRVVEREKRAVGIGAVFLGFLGAAGSTMGAASITLTVQARQLLSGIVQQQSNLLKAIEAQQHLLQLTVWGIKQLQTRVLAIERYLKDQQLLGLWGCSAKLICTTAVPWNSSWSNKSETEIWNNMTWMQWDREINNYTNTIYRLLEESQNQQEKNENDLLALDKWNSLWDWFGISNWLWYIR

SEQ ID NO: 5 - protein, 37 aa, Artificial Sequence
  Synthetic construct
SRIEGRGSGGYIPEAPRDGQAYVRKDGEWVLLSTFLG

SEQ ID NO: 6 - DNA, 111 bp, Artificial Sequence
  Synthetic construct
tcccggatcgagggcagaggcagcggaggctatattcccgaggcccccagagatggccaggcctacgtgcggaaagatggcgagtgggtgctgctgagtaccttcctgggc

SEQ ID NO: 7 - DNA, 1935 bp, Artificial Sequence
  Synthetic construct
gtgggcaacctgtgggtcaccgtgtactatggcgtgcccgtgtggcgggaagccaagaccacactgttctgtgccagcgacgccaaggcctacgaccgcgaggtgcacaatgtgtgggccacccatgcctgcgtgcccaccgatcccaacccccaggaaatcgtgctggaaaacgtgaccgagaacttcaacatgtggaagaacgacatggtggaccagatgcacgaggacatcatcagcctgtgggaccagagcctgaagccctgcgtgaagctgacccctctgtgcgtgaccctggaatgcaccgccttcaacagcagcagccacaccaacagctctatcgccatgcaggaaatgaagaactgcagcttcaatatgaccaccgagctgcgggacaagaaaaagaaggtgtccgccctgttctacaagctggacatcgtgcccctgaacaagaacggccggcagtaccggctgatcaactgcaacaccagcaccctgacccaggcctgccccaaggtgtccttcgaccccatccccatccactactgtacccctgccggctacgccatcctgaagtgcaacaacaagaccttcaacggcaccggcccctgcaacaacgtgtccaccgtgcagtgtacccacggcatcaagcccgtggtgtccacccagctgctgctgaatggcagcctggccgaggaagatatcatcatcagaagcgagaacctgaccaacaacgccaagacaatcattgtgcatctgaacgagagcgtggaaattgtgtgcatccggcccaacaacaacaccagaaagagcatccggatcggccctggccagaccttctacgccaacaacgacatcatcggcgacatccggcaggcccactgcaatatcagcaaagagaagtggaacaataccctgcaccgcgtgtggaaaaagctggtggaacacttccctaacaagaccaccatcagattcgaccggcactctggcggcgacctggaaatcaccacccacagcttcaactgtggcggcgagttcttctactgcaatacctccggcctgttcaacatcacctacaacagcaactacacctacaatgacaccaagcacaacgggaccaaagtgatcaccctgccctgcagaatcaagcagatcattaacatgtggcaggaagtgggcagggctatgtacgcccctcctatcgccggcaacatcacatgcaccagcaatatcaccggcctgctgctgaccagggacggcggcaacaatagcaccgagacagagacattcagacccggcggaggcgacatgagagacaactggcggagcgagctgtacaagtacaaggtggtggaaatcaagcccctgggaatcgcccctaccggcgccaagagaagagtggtggaacgcgagaagcgggccgtgggaatcggagccgtgttcctgggatttctgggagccgccggaagcacaatgggcgctgccagcatcaccctgacagtgcaggctagacagctgctgagcggcatcgtgcagcagcagagcaacctgctgaaggccatcgaggcccagcagcatctgctgcagctgaccgtgtgggggatcaagcagctgcagaccagagtgctggccattgagagatacctgaaggaccagcagctgctgggcctgtggggctgttctgccaagctgatctgtaccaccgccgtgccttggaacagctcctggtccaacaagagcgaaaccgagatctggaacaacatgacctggatgcagtgggacagagagatcagcaattacaccaacaccatctaccggctgctggaagagagccagaaccagcaggaaaagaacgagaacgacctgctggccctggacaagtggaactccctgtgggattggttcggcatcagcaactggctgtggtacatccgg

SEQ ID NO: 8 - DNA, 1935 bp, Artificial Sequence
  Synthetic construct
gtgggcaacctgtgggtcaccgtgtactatggcgtgcccgtgtggcgggaagccgagacaacactgttctgtgccagcgacgccaaggcctacgaccgcgaggtgcacaatgtgtgggccacccatgcctgcgtgcccaccgatcccaacccccaggaaatcgtgctggaaaacgtgaccgagaacttcaacatgtggaagaacgacatggtggaccagatgcacgaggacatcatcagcctgtgggaccagagcctgaagccctgcgtgaagctgacccctctgtgcgtgaccctggactgcaaggccttcaacagcagcagccacaccaacagctctatcgccatgcaggaaatgaagaactgcaccttcaacatcaccaccagcgtgaagggcaagcggcagcaggaacacgccctgttctacaagctggacatcgtgcccctgaacaagaacggccggcagtaccggctgatcaactgcaacaccagcaccctgacccaggcctgccccaaggtgtccttcgaccccatccccatccactactgtacccctgccggctacgccatcctgaagtgcaacaacaagaccttcaacggcaccggcccctgcaacaacgtgtccaccgtgcagtgtacccacggcatcaagcccgtggtgtccacccagctgctgctgaatggcagcctggccgaggaagatatcatcatcagaagcgagaacctgaccaacaacgccaagaccatcattgtgcatctgaacgagagcgtggaaattgtgtgcgtgcggcccaacaacaacaccagaaagagcatccggatcggccctggccagaccttctacgccaacaacgagatcatcggcgacatccggcaggcccactgcaatatcagcaaagagaagtggaacaataccctgcaccgcgtgtggaaaaagctggtggaacacttccctaacaagaccaccatcagattcgaccggcactctggcggcgacctggaaatcaccacccacagcttcaactgtggcggcgagttcttctactgcaatacctccggcctgttcaatatcacctacaacagcaactacacctacaatgacaccaagcacaacgggaccaaagtgatcaccctgccctgcagaatcaagcagatcattaacatgtggcaggaagtgggcagggctatgtacgcccctcctatcgccggcaacatcacatgcaccagcaacattaccggcctgctgctgaccagggacggcggcaacaatagcaccgagacagagacattcagacccggcggaggcgacatgagagacaactggcggagcgagctgtacaagtacaaggtggtggaaatcaagcccctgggaatcgcccctaccggcgccaagagaagagtggtggaacgcgagaagcgggccgtgggaatcggagccgtgtttctgggctttctgggagccgccggaagcacaatgggcgctgccagcatcaccctgacagtgcaggctagacagctgctgagcggcatcgtgcagcagcagagcaacctgctgaaggccatcgaggcccagcagcatctgctgcagctgaccgtgtgggggatcaagcagctgcagaccagagtgctggccattgagagatacctgaaggaccagcagctgctgggcctgtggggctgttctgccaagctgatctgtaccaccgccgtgccttggaacagctcctggtccaacaagagcgaaaccgagatctggaacaacatgacctggatgcagtgggacagagagatcagcaattacaccaacaccatctacaggctgctggaagagagccagaaccagcaggaaaagaacgagaacgacctgctggccctggacaagtggaactccctgtgggattggttcggcatcagcaactggctgtggtacatccgg

SEQ ID NO: 9 - DNA, 1935 bp, Artificial Sequence
  Synthetic construct
gtgggcaacctgtgggtcaccgtgtactatggcgtgcccgtgtggcgggaagccaagaccacactgttctgtgccagcgacgccaaggcctacgaccgcgaggtgcacaatgtgtgggccacccatgcctgcgtgcccaccgatcccaacccccaggaaatcgtgctggaaaacgtgaccgagaacttcaacatgtggaagaacgacatggtggaccagatgcacgaggacatcatcagcctgtgggaccagagcctgaagccctgcgtgaagctgacccctctgtgcgtgaccctgaactgcaccgccttcaacagcagcagccacaccaacagctctatcgccatgcaggaaatgaagaactgcagcttcaaggccaccaccgagatccgggaccggaagaaagagatgtacgccctgttctacaagctggacatcgtgcccatcaacaagaacggccggcagtaccggctgatcaactgcaacaccagcaccctgacccaggcctgccccaaggtgtccttcgaccccatccccatccactactgtacccctgccggcttcgccatcctgaagtgcaacaacaagaccttcaacggcaccggcccctgcaccaacgtgtccaccgtgcagtgtacccacggcatcaagcccgtggtgtccacccagctgctgctgaatggcagcctggccgaggaagatatcatcatcagaagcgagaacctgaccaacaacgccaagacaatcatcgtgcacctgaacgagagcgtggaaatcaattgcaccagacccggcaacaacaccagaaagagcatccggatcggccctggccagaccttctacgccaacaacgacatcatcggcgacatccggcaggcccactgcaacatctctgaggccaagtggaacaacacactgcaccaggtggccaagaaactggtggaacacttccctaacaagaccaccatcagattcgaccggcactctggcggcgacctggaaatcaccacccacagcttcaactgtggcggcgagttcttctactgcaatacctccggcctgttcaacatcacctacaacagcaactacacctacaatgacaccaagcacaacgggaccaaagtgatcaccctgccctgcagaatcaagcagatcattaacatgtggcaggaagtgggcagggctatgtatgcccctcctatcgccggcaacattacctgcaccagcaatatcaccggcctgctgctgaccagggacggcggcaacaatagcaccgagacagagacattccggcctggcggcggagacatgagagacaattggcggagcgagctgtacaagtacaaggtggtggaaatcaagcccctgggaatcgcccctaccggcgccaagagaagagtggtggaacgcgagaagcgggccgtgggaatcggagccgtgttcctgggatttctgggagccgccggaagcacaatgggcgctgccagcatcaccctgacagtgcaggctagacagctgctgagcggcatcgtgcagcagcagagcaacctgctgaaggccatcgaggcccagcagcatctgctgcagctgaccgtgtgggggatcaagcagctgcagaccagagtgctggccattgagagatacctgaaggaccagcagctgctgggcctgtggggctgttctgccaagctgatctgtaccaccgccgtgccttggaacagctcctggtccaacaagagcgaaaccgagatctggaacaatatgacatggatgcagtgggaccgcgagatcaacaattacaccaacaccatctaccggctgctggaagagagccagaaccagcaggaaaagaacgagaacgacctgctggccctggacaagtggaactccctgtgggattggttcggcatcagcaactggctgtggtacatccgc

SEQ ID NO: 10 - DNA, 1935 bp, Artificial Sequence
  Synthetic construct
gtgggcaacctgtgggtcaccgtgtactatggcgtgcccgtgtggcgggaagccaagaccacactgttctgtgccagcgacgccaaggcctacgaccgcgaggtgcacaatgtgtgggccacccatgcctgcgtgcccaccgatcccaacccccaggaaatcgtgctggaaaacgtgaccgagaacttcaacatgtggaagaacgacatggtggaccagatgcacgaggacatcatcagcctgtgggaccagagcctgaagccctgcgtgaagctgacccctctgtgcgtgaccctgaactgcaccgccttcaacagcagcagccacaccaacagctctatcgccatgcaggaaatgaagaactgcagcttcaacgccaccaccgagatccgggaccggaagaaagagatgtacgccctgttctacaagctggacatcgtgcccatcaacaagaacggccggcagtaccggctgatcaactgcaacaccagcaccctgacccaggcctgccccaaggtgtccttcgaccccatccccatccactactgtacccctgccggcttcgccatcctgaagtgcaacaacaagaccttcaacggcaccggcccctgcaccaacgtgtccaccgtgcagtgtacccacggcatcaagcccgtggtgtccacccagctgctgctgaatggcagcctggccgaggaagatatcatcatcagaagcgagaacctgagcaacaacgccaagacaatcatcgtgcacctgaacgagagcgtggaaatcacctgtatccggcccagcaacaacaccagaaagagcgtgcggatcggccctggccagaccttctacgccaacaacgacatcatcggcaacatccggaaggcctactgcgagatcaacgagacaaagtggaacaacacactgcataatgtgtccaagaaactggtggaacacttccctaacaagaccaccatcagattcgaccggcactctggcggcgacctggaaattaccacccacagcttcaattgtggcggcgagttcttctactgcaatacctccggcctgttcaacatcagctacaacagcaactacacctacaacgacaccaagcacaacgggaccaaagtgatcaccctgccctgccggatcaagcagatcattaacatgtggcaggaagtgggcagggctatgtatgcccctcctatcgccggcaacattacctgcacctccaacatcaccggcctgctgctgaccagagatggcggcaacaactccaccgagacagagacattcagacccggcggaggcgacatgagagacaactggcggagcgagctgtacaagtacaaggtggtggaaatcaagcccctgggaatcgcccctaccggcgccaagagaagagtggtggaacgcgagaagcgggccgtgggaatcggagccgtgttcctgggatttctgggagccgccggaagcacaatgggcgctgccagcatcaccctgacagtgcaggctagacagctgctgagcggcatcgtgcagcagcagagcaacctgctgaaggccatcgaggcccagcagcatctgctgcagctgaccgtgtggggaatcaagcagctgcagacacgggtgctggccattgagagatacctgaaggaccagcagctgctgggcctgtggggctgttctgccaagctgatctgtaccaccgccgtgccctggaacagctcctggtccaacaagagcgaaaccgagatctggaacaatatgacctggatgcagtgggaccgggaaatcaacaattacaccaacaccatctaccggctgctggaagagagccagaaccagcaggaaaagaacgagaacgacctgctggccctggacaagtggaactccctgtgggattggttcggcatcagcaactggctgtggtacatccgc

SEQ ID NO: 11 - protein, 688 aa, Artificial Sequence
  Synthetic construct
VGNLWVTVYYGVPVWREAKTTLFCASDAKAYDREVHNVWATHACVPTDPNPQEIVLENVTENFNMWKNDMVDQMHEDIISLWDQSLKPCVKLTPLCVTLECTAFNSSSHTNSSIAMQEMKNCSFNMTTELRDKKKKVSALFYKLDIVPLNKNGRQYRLINCNTSTLTQACPKVSFDPIPIHYCTPAGYAILKCNNKTFNGTGPCNNVSTVQCTHGIKPVVSTQLLLNGSLAEEDIIIRSENLTNNAKTIIVHLNESVEIVCIRPNNNTRKSIRIGPGQTFYANNDIIGDIRQAHCNISKEKWNNTLHRVWKKLVEHFPNKTTIRFDRHSGGDLEITTHSFNCGGEFFYCNTSGLFNITYNSNYTYNDTKHNGTKVITLPCRIKQIINMWQEVGRAMYAPPIAGNITCTSNITGLLLTRDGGNNSTETETFRPGGGDMRDNWRSELYKYKVVEIKPLGIAPTGAKRRVVEREKRAVGIGAVFLGFLGAAGSTMGAASITLTVQARQLLSGIVQQQSNLLKAIEAQQHLLQLTVWGIKQLQTRVLAIERYLKDQQLLGLWGCSAKLICTTAVPWNSSWSNKSETEIWNNMTWMQWDREISNYTNTIYRLLEESQNQQEKNENDLLALDKWNSLWDWFGISNWLWYIRSRIEGRGSGGYIPEAPRDGQAYVRKDGEWVLLSTFLGHHHHHH

SEQ ID NO: 12 - protein, 688 aa, Artificial Sequence
  Synthetic construct
VGNLWVTVYYGVPVWREAETTLFCASDAKAYDREVHNVWATHACVPTDPNPQEIVLENVTENFNMWKNDMVDQMHEDIISLWDQSLKPCVKLTPLCVTLDCKAFNSSSHTNSSIAMQEMKNCTFNITTSVKGKRQQEHALFYKLDIVPLNKNGRQYRLINCNTSTLTQACPKVSFDPIPIHYCTPAGYAILKCNNKTFNGTGPCNNVSTVQCTHGIKPVVSTQLLLNGSLAEEDIIIRSENLTNNAKTIIVHLNESVEIVCVRPNNNTRKSIRIGPGQTFYANNEIIGDIRQAHCNISKEKWNNTLHRVWKKLVEHFPNKTTIRFDRHSGGDLEITTHSFNCGGEFFYCNTSGLFNITYNSNYTYNDTKHNGTKVITLPCRIKQIINMWQEVGRAMYAPPIAGNITCTSNITGLLLTRDGGNNSTETETFRPGGGDMRDNWRSELYKYKVVEIKPLGIAPTGAKRRVVEREKRAVGIGAVFLGFLGAAGSTMGAASITLTVQARQLLSGIVQQQSNLLKAIEAQQHLLQLTVWGIKQLQTRVLAIERYLKDQQLLGLWGCSAKLICTTAVPWNSSWSNKSETEIWNNMTWMQWDREISNYTNTIYRLLEESQNQQEKNENDLLALDKWNSLWDWFGISNWLWYIRSRIEGRGSGGYIPEAPRDGQAYVRKDGEWVLLSTFLGHHHHHH

SEQ ID NO: 13 - protein, 688 aa, Artificial Sequence
  Synthetic construct
VGNLWVTVYYGVPVWREAKTTLFCASDAKAYDREVHNVWATHACVPTDPNPQEIVLENVTENFNMWKNDMVDQMHEDIISLWDQSLKPCVKLTPLCVTLNCTAFNSSSHTNSSIAMQEMKNCSFKATTEIRDRKKEMYALFYKLDIVPINKNGRQYRLINCNTSTLTQACPKVSFDPIPIHYCTPAGFAILKCNNKTFNGTGPCTNVSTVQCTHGIKPVVSTQLLLNGSLAEEDIIIRSENLTNNAKTIIVHLNESVEINCTRPGNNTRKSIRIGPGQTFYANNDIIGDIRQAHCNISEAKWNNTLHQVAKKLVEHFPNKTTIRFDRHSGGDLEITTHSFNCGGEFFYCNTSGLFNITYNSNYTYNDTKHNGTKVITLPCRIKQIINMWQEVGRAMYAPPIAGNITCTSNITGLLLTRDGGNNSTETETFRPGGGDMRDNWRSELYKYKVVEIKPLGIAPTGAKRRVVEREKRAVGIGAVFLGFLGAAGSTMGAASITLTVQARQLLSGIVQQQSNLLKAIEAQQHLLQLTVWGIKQLQTRVLAIERYLKDQQLLGLWGCSAKLICTTAVPWNSSWSNKSETEIWNNMTWMQWDREINNYTNTIYRLLEESQNQQEKNENDLLALDKWNSLWDWFGISNWLWYIRSRIEGRGSGGYIPEAPRDGQAYVRKDGEWVLLSTFLGHHHHHH

SEQ ID NO: 14 - protein, 688 aa, Artificial Sequence
  Synthetic construct
VGNLWVTVYYGVPVWREAKTTLFCASDAKAYDREVHNVWATHACVPTDPNPQEIVLENVTENFNMWKNDMVDQMHEDIISLWDQSLKPCVKLTPLCVTLNCTAFNSSSHTNSSIAMQEMKNCSFNATTEIRDRKKEMYALFYKLDIVPINKNGRQYRLINCNTSTLTQACPKVSFDPIPIHYCTPAGFAILKCNNKTFNGTGPCTNVSTVQCTHGIKPVVSTQLLLNGSLAEEDIIIRSENLSNNAKTIIVHLNESVEITCIRPSNNTRKSVRIGPGQTFYANNDIIGNIRKAYCEINETKWNNTLHNVSKKLVEHFPNKTTIRFDRHSGGDLEITTHSFNCGGEFFYCNTSGLFNISYNSNYTYNDTKHNGTKVITLPCRIKQIINMWQEVGRAMYAPPIAGNITCTSNITGLLLTRDGGNNSTETETFRPGGGDMRDNWRSELYKYKVVEIKPLGIAPTGAKRRVVEREKRAVGIGAVFLGFLGAAGSTMGAASITLTVQARQLLSGIVQQQSNLLKAIEAQQHLLQLTVWGIKQLQTRVLAIERYLKDQQLLGLWGCSAKLICTTAVPWNSSWSNKSETEIWNNMTWMQWDREINNYTNTIYRLLEESQNQQEKNENDLLALDKWNSLWDWFGISNWLWYIRSRIEGRGSGGYIPEAPRDGQAYVRKDGEWVLLSTFLGHHHHHH

SEQ ID NO: 15 - DNA, 1989 bp, Human immunodeficiency virus type 1
gtgggcaacctgtgggtgacagtgtactacggcgtgcccgtgtggcgcgaggccaagaccaccctgttctgcgccagcgacgccaaggcctacgaccgcgaggtgcacaacgtgtgggccacccacgcctgcgtgccaacagaccccaacccccaggaaatcgtcctggaaaacgtgaccgagaacttcaacatgtggaagaacgacatggtggaccagatgcacgaggacatcatcagcctgtgggaccagagcctgaagccctgcgtgaagctgacccctctgtgcgtgaccctgaactgcaccaacgtgaccagcagcgccgccaatgtgacctctaacgtgaccaacgacgccaacaacgcctccaacgccaacggccggaacgtgatcaacgaggacatgcagaactgcagcttcaacgccaccaccgagatccgggaccggaagaaagagatgtacgccctgttctacaagctggacatcgtgcccctggacggcgagaagtccgacaaccggtacagactgatcaactgcaacaccagcaccctgacccaggcctgccccaaggtgtccttcgaccccatccccatccactactgcacccctgccggcttcgccatcctgaagtgcaacaacaagaccttcaacggcaccggcccctgcaacaacgtgtccaccgtgcagtgcacccacggcatcaagcccgtggtgtccacccagctgctgctgaacggcagcctggccgaggaagatatcatcatcagaagcgagaacctgaccaacaatgccaagaccatcatcgtgcacctgaacgagagcgtggaaatcgtgtgcacccggcccaacaacaacaccagaaagagcatccggatcggccctggccagaccttctacgccaacaatgacatcatcggcgacatccggcaggcccactgcaacatcagcgaggaaaagtggaacaacaccctgcaccgcgtgtggaagaaactggtggaacacttccccaacaagaccaccatcagattcgaccggcactctggcggcgacctggaaatcaccacccacagcttcaactgtggcggcgagttcttctactgcaataccagcggcctgttcaacatcacctacaacagcaactacacctacaacgacaccaagcacaacggcaccaaagtgatcaccctgccctgccggatcaagcagatcatcaatatgtggcaagaagtgggcagagctatgtacgcccctcctatcgccggcaacatcacatgcaccagcaacatcaccggcctgctgctgacccgggacggcggcaacaacagcaccgagacagagacattcagacccggcggaggcgacatgcgggacaattggcggagcgagctgtacaagtacaaggtggtggaaatcaagcccctgggaatcgcccccaccggcgccaagagaagagtggtggaacgcgagaagcgggccgtgggcatcggcgccgtgtttctgggctttctgggagccgccggaagcacaatgggcgctgcctccatcaccctgaccgtgcaggccagacagctgctgagcggcatcgtgcagcagcagagcaacctgctcaaggccatcgaggcccagcagcatctgctgcagctgaccgtgtggggcatcaagcagctgcagacccgggtgctggccatcgagagatacctgaaggaccagcagctcctgggcctgtggggctgcagcgccaagctgatctgcaccaccgccgtgccctggaacagcagctggtccaacaagagcgaaaccgagatctggaacaacatgacctggatgcagtgggaccgcgagatcaacaactacaccaacaccatctaccggctgctggaagagagccagaaccagcaggaaaagaacgagaacgacctgctggccctggacaagtggaactccctgtgggattggttcggcatcagcaactggctgtggtacatcaga

SEQ ID NO: 16 - protein, 663 aa, Human immunodeficiency virus type 1
VGNLWVTVYYGVPVWREAKTTLFCASDAKAYDREVHNVWATHACVPTDPNPQEIVLENVTENFNMWKNDMVDQMHEDIISLWDQSLKPCVKLTPLCVTLNCTNVTSSAANVTSNVTNDANNASNANGRNVINEDMQNCSFNATTEIRDRKKEMYALFYKLDIVPLDGEKSDNRYRLINCNTSTLTQACPKVSFDPIPIHYCTPAGFAILKCNNKTFNGTGPCNNVSTVQCTHGIKPVVSTQLLLNGSLAEEDIIIRSENLTNNAKTIIVHLNESVEIVCTRPNNNTRKSIRIGPGQTFYANNDIIGDIRQAHCNISEEKWNNTLHRVWKKLVEHFPNKTTIRFDRHSGGDLEITTHSFNCGGEFFYCNTSGLFNITYNSNYTYNDTKHNGTKVITLPCRIKQIINMWQEVGRAMYAPPIAGNITCTSNITGLLLTRDGGNNSTETETFRPGGGDMRDNWRSELYKYKVVEIKPLGIAPTGAKSSVVERAKSAVGIGAVFLGFLGAAGSTMGAASITLTVQARQLLSGIVQQQSNLLKAIEAQQHLLQLTVWGIKQLQTRVLAIERYLKDQQLLGLWGCSAKLICTTAVPWNSSWSNKSETEIWNNMTWMQWDREINNYTNTIYRLLEESQNQQEKNENDLLALDKWNSLWDWFGISNWLWYIR

SEQ ID NO: 17 - protein, 29 aa, Artificial Sequence
  Synthetic construct
MRVRGIQRNCQHLWRWGTLILGMLMICSA

SEQ ID NO: 18 - DNA, 87 bp, Artificial Sequence
  Synthetic construct
atgagagtgcggggcatccagcggaattgccagcacctgtggcgctggggcacactgatcctgggcatgctgatgatctgcagcgcc

SEQ ID NO: 19 - protein, 717 aa, Artificial Sequence
  Synthetic construct
MRVRGIQRNCQHLWRWGTLILGMLMICSAVGNLWVTVYYGVPVWREAKTTLFCASDAKAYDREVHNVWATHACVPTDPNPQEIVLENVTENFNMWKNDMVDQMHEDIISLWDQSLKPCVKLTPLCVTLECTAFNSSSHTNSSIAMQEMKNCSFNMTTELRDKKKKVSALFYKLDIVPLNKNGRQYRLINCNTSTLTQACPKVSFDPIPIHYCTPAGYAILKCNNKTFNGTGPCNNVSTVQCTHGIKPVVSTQLLLNGSLAEEDIIIRSENLTNNAKTIIVHLNESVEIVCIRPNNNTRKSIRIGPGQTFYANNDIIGDIRQAHCNISKEKWNNTLHRVWKKLVEHFPNKTTIRFDRHSGGDLEITTHSFNCGGEFFYCNTSGLFNITYNSNYTYNDTKHNGTKVITLPCRIKQIINMWQEVGRAMYAPPIAGNITCTSNITGLLLTRDGGNNSTETETFRPGGGDMRDNWRSELYKYKVVEIKPLGIAPTGAKRRVVEREKRAVGIGAVFLGFLGAAGSTMGAASITLTVQARQLLSGIVQQQSNLLKAIEAQQHLLQLTVWGIKQLQTRVLAIERYLKDQQLLGLWGCSAKLICTTAVPWNSSWSNKSETEIWNNMTWMQWDREISNYTNTIYRLLEESQNQQEKNENDLLALDKWNSLWDWFGISNWLWYIRSRIEGRGSGGYIPEAPRDGQAYVRKDGEWVLLSTFLGHHHHHH

SEQ ID NO: 20 - protein, 717 aa, Artificial Sequence
  Synthetic construct
MRVRGIQRNCQHLWRWGTLILGMLMICSAVGNLWVTVYYGVPVWREAETTLFCASDAKAYDREVHNVWATHACVPTDPNPQEIVLENVTENFNMWKNDMVDQMHEDIISLWDQSLKPCVKLTPLCVTLDCKAFNSSSHTNSSIAMQEMKNCTFNITTSVKGKRQQEHALFYKLDIVPLNKNGRQYRLINCNTSTLTQACPKVSFDPIPIHYCTPAGYAILKCNNKTFNGTGPCNNVSTVQCTHGIKPVVSTQLLLNGSLAEEDIIIRSENLTNNAKTIIVHLNESVEIVCVRPNNNTRKSIRIGPGQTFYANNEIIGDIRQAHCNISKEKWNNTLHRVWKKLVEHFPNKTTIRFDRHSGGDLEITTHSFNCGGEFFYCNTSGLFNITYNSNYTYNDTKHNGTKVITLPCRIKQIINMWQEVGRAMYAPPIAGNITCTSNITGLLLTRDGGNNSTETETFRPGGGDMRDNWRSELYKYKVVEIKPLGIAPTGAKRRVVEREKRAVGIGAVFLGFLGAAGSTMGAASITLTVQARQLLSGIVQQQSNLLKAIEAQQHLLQLTVWGIKQLQTRVLAIERYLKDQQLLGLWGCSAKLICTTAVPWNSSWSNKSETEIWNNMTWMQWDREISNYTNTIYRLLEESQNQQEKNENDLLALDKWNSLWDWFGISNWLWYIRSRIEGRGSGGYIPEAPRDGQAYVRKDGEWVLLSTFLGHHHHHH

SEQ ID NO: 21 - protein, 717 aa, Artificial Sequence
  Synthetic construct
MRVRGIQRNCQHLWRWGTLILGMLMICSAVGNLWVTVYYGVPVWREAKTTLFCASDAKAYDREVHNVWATHACVPTDPNPQEIVLENVTENFNMWKNDMVDQMHEDIISLWDQSLKPCVKLTPLCVTLNCTAFNSSSHTNSSIAMQEMKNCSFKATTEIRDRKKEMYALFYKLDIVPINKNGRQYRLINCNTSTLTQACPKVSFDPIPIHYCTPAGFAILKCNNKTFNGTGPCTNVSTVQCTHGIKPVVSTQLLLNGSLAEEDIIIRSENLTNNAKTIIVHLNESVEINCTRPGNNTRKSIRIGPGQTFYANNDIIGDIRQAHCNISEAKWNNTLHQVAKKLVEHFPNKTTIRFDRHSGGDLEITTHSFNCGGEFFYCNTSGLFNITYNSNYTYNDTKHNGTKVITLPCRIKQIINMWQEVGRAMYAPPIAGNITCTSNITGLLLTRDGGNNSTETETFRPGGGDMRDNWRSELYKYKVVEIKPLGIAPTGAKRRVVEREKRAVGIGAVFLGFLGAAGSTMGAASITLTVQARQLLSGIVQQQSNLLKAIEAQQHLLQLTVWGIKQLQTRVLAIERYLKDQQLLGLWGCSAKLICTTAVPWNSSWSNKSETEIWNNMTWMQWDREINNYTNTIYRLLEESQNQQEKNENDLLALDKWNSLWDWFGISNWLWYIRSRIEGRGSGGYIPEAPRDGQAYVRKDGEWVLLSTFLGHHHHHH

SEQ ID NO: 22 - protein, 717 aa, Artificial Sequence
  Synthetic construct
MRVRGIQRNCQHLWRWGTLILGMLMICSAVGNLWVTVYYGVPVWREAKTTLFCASDAKAYDREVHNVWATHACVPTDPNPQEIVLENVTENFNMWKNDMVDQMHEDIISLWDQSLKPCVKLTPLCVTLNCTAFNSSSHTNSSIAMQEMKNCSFNATTEIRDRKKEMYALFYKLDIVPINKNGRQYRLINCNTSTLTQACPKVSFDPIPIHYCTPAGFAILKCNNKTFNGTGPCTNVSTVQCTHGIKPVVSTQLLLNGSLAEEDIIIRSENLSNNAKTIIVHLNESVEITCIRPSNNTRKSVRIGPGQTFYANNDIIGNIRKAYCEINETKWNNTLHNVSKKLVEHFPNKTTIRFDRHSGGDLEITTHSFNCGGEFFYCNTSGLFNISYNSNYTYNDTKHNGTKVITLPCRIKQIINMWQEVGRAMYAPPIAGNITCTSNITGLLLTRDGGNNSTETETFRPGGGDMRDNWRSELYKYKVVEIKPLGIAPTGAKRRVVEREKRAVGIGAVFLGFLGAAGSTMGAASITLTVQARQLLSGIVQQQSNLLKAIEAQQHLLQLTVWGIKQLQTRVLAIERYLKDQQLLGLWGCSAKLICTTAVPWNSSWSNKSETEIWNNMTWMQWDREINNYTNTIYRLLEESQNQQEKNENDLLALDKWNSLWDWFGISNWLWYIRSRIEGRGSGGYIPEAPRDGQAYVRKDGEWVLLSTFLGHHHHHH

SEQ ID NO: 23 - protein, 731 aa, Human immunodeficiency virus type 1
MDAMKRGLCCVLLLCGAVFVSPSASVGNLWVTVYYGVPVWREAKTTLFCASDAKAYDREVHNVWATHACVPTDPNPQEIVLENVTENFNMWKNDMVDQMHEDIISLWDQSLKPCVKLTPLCVTLNCTNVTSSAANVTSNVTNDANNASNANGRNVINEDMQNCSFNATTEIRDRKKEMYALFYKLDIVPLDGEKSDNRYRLINCNTSTLTQACPKVSFDPIPIHYCTPAGFAILKCNNKTFNGTGPCNNVSTVQCTHGIKPVVSTQLLLNGSLAEEDIIIRSENLTNNAKTIIVHLNESVEIVCTRPNNNTRKSIRIGPGQTFYANNDIIGDIRQAHCNISEEKWNNTLHRVWKKLVEHFPNKTTIRFDRHSGGDLEITTHSFNCGGEFFYCNTSGLFNITYNSNYTYNDTKHNGTKVITLPCRIKQIINMWQEVGRAMYAPPIAGNITCTSNITGLLLTRDGGNNSTETETFRPGGGDMRDNWRSELYKYKVVEIKPLGIAPTGAKSSVVERAKSAVGIGAVFLGFLGAAGSTMGAASITLTVQARQLLSGIVQQQSNLLKAIEAQQHLLQLTVWGIKQLQTRVLAIERYLKDQQLLGLWGCSAKLICTTAVPWNSSWSNKSETEIWNNMTWMQWDREINNYTNTIYRLLEESQNQQEKNENDLLALDKWNSLWDWFGISNWLWYIRSRIEGRGSGGYIPEAPRDGQAYVRKDGEWVLLSTFLGHHHHHH

SEQ ID NO: 24 - DNA, 2205 bp, Human immunodeficiency virus type 1
atgagagtgcggggcatccagcggaactgccagcatctgtggcgctggggcaccctgatcctgggcatgctgatgatctgcagcgccgtgggcaacctgtgggtgacagtgtactacggcgtgcccgtgtggcgcgaggccaagaccaccctgttctgcgccagcgacgccaaggcctacgaccgcgaggtgcacaacgtgtgggccacccacgcctgcgtgccaacagaccccaacccccaggaaatcgtcctggaaaacgtgaccgagaacttcaacatgtggaagaacgacatggtggaccagatgcacgaggacatcatcagcctgtgggaccagagcctgaagccctgcgtgaagctgacccctctgtgcgtgaccctgaactgcaccaacgtgaccagcagcgccgccaatgtgacctctaacgtgaccaacgacgccaacaacgcctccaacgccaacggccggaacgtgatcaacgaggacatgcagaactgcagcttcaacgccaccaccgagatccgggaccggaagaaagagatgtacgccctgttctacaagctggacatcgtgcccctggacggcgagaagtccgacaaccggtacagactgatcaactgcaacaccagcaccctgacccaggcctgccccaaggtgtccttcgaccccatccccatccactactgcacccctgccggcttcgccatcctgaagtgcaacaacaagaccttcaacggcaccggcccctgcaacaacgtgtccaccgtgcagtgcacccacggcatcaagcccgtggtgtccacccagctgctgctgaacggcagcctggccgaggaagatatcatcatcagaagcgagaacctgaccaacaatgccaagaccatcatcgtgcacctgaacgagagcgtggaaatcgtgtgcacccggcccaacaacaacaccagaaagagcatccggatcggccctggccagaccttctacgccaacaatgacatcatcggcgacatccggcaggcccactgcaacatcagcgaggaaaagtggaacaacaccctgcaccgcgtgtggaagaaactggtggaacacttccccaacaagaccaccatcagattcgaccggcactctggcggcgacctggaaatcaccacccacagcttcaactgtggcggcgagttcttctactgcaataccagcggcctgttcaacatcacctacaacagcaactacacctacaacgacaccaagcacaacggcaccaaagtgatcaccctgccctgccggatcaagcagatcatcaatatgtggcaagaagtgggcagagctatgtacgcccctcctatcgccggcaacatcacatgcaccagcaacatcaccggcctgctgctgacccgggacggcggcaacaacagcaccgagacagagacattcagacccggcggaggcgacatgcgggacaattggcggagcgagctgtacaagtacaaggtggtggaaatcaagcccctgggaatcgcccccaccggcgccaagagaagagtggtggaacgcgagaagcgggccgtgggcatcggcgccgtgtttctgggctttctgggagccgccggaagcacaatgggcgctgcctccatcaccctgaccgtgcaggccagacagctgctgagcggcatcgtgcagcagcagagcaacctgctcaaggccatcgaggcccagcagcatctgctgcagctgaccgtgtggggcatcaagcagctgcagacccgggtgctggccatcgagagatacctgaaggaccagcagctcctgggcctgtggggctgcagcgccaagctgatctgcaccaccgccgtgccctggaacagcagctggtccaacaagagcgaaaccgagatctggaacaacatgacctggatgcagtgggaccgcgagatcaacaactacaccaacaccatctaccggctgctggaagagagccagaaccagcaggaaaagaacgagaacgacctgctggccctggacaagtggaactccctgtgggattggttcggcatcagcaactggctgtggtacatcagaagccggatcgagggcagaggcagcggcggctatatccccgaggcccctagagatggccaggcctacgtgcggaaggacggcgagtgggtgctgctgagcaccttcctgggccaccaccaccatcaccac

SEQ ID NO: 25 - DNA, 2151 bp, Artificial Sequence
  Synthetic construct
atgagagtgcggggcatccagcggaattgccagcacctgtggcgctggggcacactgatcctgggcatgctgatgatctgcagcgccgtgggcaacctgtgggtcaccgtgtactatggcgtgcccgtgtggcgggaagccaagaccacactgttctgtgccagcgacgccaaggcctacgaccgcgaggtgcacaatgtgtgggccacccatgcctgcgtgcccaccgatcccaacccccaggaaatcgtgctggaaaacgtgaccgagaacttcaacatgtggaagaacgacatggtggaccagatgcacgaggacatcatcagcctgtgggaccagagcctgaagccctgcgtgaagctgacccctctgtgcgtgaccctggaatgcaccgccttcaacagcagcagccacaccaacagctctatcgccatgcaggaaatgaagaactgcagcttcaatatgaccaccgagctgcgggacaagaaaaagaaggtgtccgccctgttctacaagctggacatcgtgcccctgaacaagaacggccggcagtaccggctgatcaactgcaacaccagcaccctgacccaggcctgccccaaggtgtccttcgaccccatccccatccactactgtacccctgccggctacgccatcctgaagtgcaacaacaagaccttcaacggcaccggcccctgcaacaacgtgtccaccgtgcagtgtacccacggcatcaagcccgtggtgtccacccagctgctgctgaatggcagcctggccgaggaagatatcatcatcagaagcgagaacctgaccaacaacgccaagacaatcattgtgcatctgaacgagagcgtggaaattgtgtgcatccggcccaacaacaacaccagaaagagcatccggatcggccctggccagaccttctacgccaacaacgacatcatcggcgacatccggcaggcccactgcaatatcagcaaagagaagtggaacaataccctgcaccgcgtgtggaaaaagctggtggaacacttccctaacaagaccaccatcagattcgaccggcactctggcggcgacctggaaatcaccacccacagcttcaactgtggcggcgagttcttctactgcaatacctccggcctgttcaacatcacctacaacagcaactacacctacaatgacaccaagcacaacgggaccaaagtgatcaccctgccctgcagaatcaagcagatcattaacatgtggcaggaagtgggcagggctatgtacgcccctcctatcgccggcaacatcacatgcaccagcaatatcaccggcctgctgctgaccagggacggcggcaacaatagcaccgagacagagacattcagacccggcggaggcgacatgagagacaactggcggagcgagctgtacaagtacaaggtggtggaaatcaagcccctgggaatcgcccctaccggcgccaagagaagagtggtggaacgcgagaagcgggccgtgggaatcggagccgtgttcctgggatttctgggagccgccggaagcacaatgggcgctgccagcatcaccctgacagtgcaggctagacagctgctgagcggcatcgtgcagcagcagagcaacctgctgaaggccatcgaggcccagcagcatctgctgcagctgaccgtgtgggggatcaagcagctgcagaccagagtgctggccattgagagatacctgaaggaccagcagctgctgggcctgtggggctgttctgccaagctgatctgtaccaccgccgtgccttggaacagctcctggtccaacaagagcgaaaccgagatctggaacaacatgacctggatgcagtgggacagagagatcagcaattacaccaacaccatctaccggctgctggaagagagccagaaccagcaggaaaagaacgagaacgacctgctggccctggacaagtggaactccctgtgggattggttcggcatcagcaactggctgtggtacatccggtcccggatcgagggcagaggcagcggaggctatattcccgaggcccccagagatggccaggcctacgtgcggaaagatggcgagtgggtgctgctgagtaccttcctgggccaccatcaccaccaccac

SEQ ID NO: 26 - DNA, 2151 bp, Artificial Sequence
  Synthetic construct
atgagagtgcggggcatccagcggaattgccagcacctgtggcgctggggcacactgatcctgggcatgctgatgatctgcagcgccgtgggcaacctgtgggtcaccgtgtactatggcgtgcccgtgtggcgggaagccgagacaacactgttctgtgccagcgacgccaaggcctacgaccgcgaggtgcacaatgtgtgggccacccatgcctgcgtgcccaccgatcccaacccccaggaaatcgtgctggaaaacgtgaccgagaacttcaacatgtggaagaacgacatggtggaccagatgcacgaggacatcatcagcctgtgggaccagagcctgaagccctgcgtgaagctgacccctctgtgcgtgaccctggactgcaaggccttcaacagcagcagccacaccaacagctctatcgccatgcaggaaatgaagaactgcaccttcaacatcaccaccagcgtgaagggcaagcggcagcaggaacacgccctgttctacaagctggacatcgtgcccctgaacaagaacggccggcagtaccggctgatcaactgcaacaccagcaccctgacccaggcctgccccaaggtgtccttcgaccccatccccatccactactgtacccctgccggctacgccatcctgaagtgcaacaacaagaccttcaacggcaccggcccctgcaacaacgtgtccaccgtgcagtgtacccacggcatcaagcccgtggtgtccacccagctgctgctgaatggcagcctggccgaggaagatatcatcatcagaagcgagaacctgaccaacaacgccaagaccatcattgtgcatctgaacgagagcgtggaaattgtgtgcgtgcggcccaacaacaacaccagaaagagcatccggatcggccctggccagaccttctacgccaacaacgagatcatcggcgacatccggcaggcccactgcaatatcagcaaagagaagtggaacaataccctgcaccgcgtgtggaaaaagctggtggaacacttccctaacaagaccaccatcagattcgaccggcactctggcggcgacctggaaatcaccacccacagcttcaactgtggcggcgagttcttctactgcaatacctccggcctgttcaatatcacctacaacagcaactacacctacaatgacaccaagcacaacgggaccaaagtgatcaccctgccctgcagaatcaagcagatcattaacatgtggcaggaagtgggcagggctatgtacgcccctcctatcgccggcaacatcacatgcaccagcaacattaccggcctgctgctgaccagggacggcggcaacaatagcaccgagacagagacattcagacccggcggaggcgacatgagagacaactggcggagcgagctgtacaagtacaaggtggtggaaatcaagcccctgggaatcgcccctaccggcgccaagagaagagtggtggaacgcgagaagcgggccgtgggaatcggagccgtgtttctgggctttctgggagccgccggaagcacaatgggcgctgccagcatcaccctgacagtgcaggctagacagctgctgagcggcatcgtgcagcagcagagcaacctgctgaaggccatcgaggcccagcagcatctgctgcagctgaccgtgtgggggatcaagcagctgcagaccagagtgctggccattgagagatacctgaaggaccagcagctgctgggcctgtggggctgttctgccaagctgatctgtaccaccgccgtgccttggaacagctcctggtccaacaagagcgaaaccgagatctggaacaacatgacctggatgcagtgggacagagagatcagcaattacaccaacaccatctacaggctgctggaagagagccagaaccagcaggaaaagaacgagaacgacctgctggccctggacaagtggaactccctgtgggattggttcggcatcagcaactggctgtggtacatccggtcccggatcgagggcagaggcagcggaggctatattcccgaggcccccagagatggccaggcctacgtgcggaaagatggcgagtgggtgctgctgagtaccttcctgggccaccatcaccatcatcac

SEQ ID NO: 27 - DNA, 2151 bp, Artificial Sequence
  Synthetic construct
atgagagtgcggggcatccagcggaattgccagcacctgtggcgctggggcacactgatcctgggcatgctgatgatctgcagcgccgtgggcaacctgtgggtcaccgtgtactatggcgtgcccgtgtggcgggaagccaagaccacactgttctgtgccagcgacgccaaggcctacgaccgcgaggtgcacaatgtgtgggccacccatgcctgcgtgcccaccgatcccaacccccaggaaatcgtgctggaaaacgtgaccgagaacttcaacatgtggaagaacgacatggtggaccagatgcacgaggacatcatcagcctgtgggaccagagcctgaagccctgcgtgaagctgacccctctgtgcgtgaccctgaactgcaccgccttcaacagcagcagccacaccaacagctctatcgccatgcaggaaatgaagaactgcagcttcaaggccaccaccgagatccgggaccggaagaaagagatgtacgccctgttctacaagctggacatcgtgcccatcaacaagaacggccggcagtaccggctgatcaactgcaacaccagcaccctgacccaggcctgccccaaggtgtccttcgaccccatccccatccactactgtacccctgccggcttcgccatcctgaagtgcaacaacaagaccttcaacggcaccggcccctgcaccaacgtgtccaccgtgcagtgtacccacggcatcaagcccgtggtgtccacccagctgctgctgaatggcagcctggccgaggaagatatcatcatcagaagcgagaacctgaccaacaacgccaagacaatcatcgtgcacctgaacgagagcgtggaaatcaattgcaccagacccggcaacaacaccagaaagagcatccggatcggccctggccagaccttctacgccaacaacgacatcatcggcgacatccggcaggcccactgcaacatctctgaggccaagtggaacaacacactgcaccaggtggccaagaaactggtggaacacttccctaacaagaccaccatcagattcgaccggcactctggcggcgacctggaaatcaccacccacagcttcaactgtggcggcgagttcttctactgcaatacctccggcctgttcaacatcacctacaacagcaactacacctacaatgacaccaagcacaacgggaccaaagtgatcaccctgccctgcagaatcaagcagatcattaacatgtggcaggaagtgggcagggctatgtatgcccctcctatcgccggcaacattacctgcaccagcaatatcaccggcctgctgctgaccagggacggcggcaacaatagcaccgagacagagacattccggcctggcggcggagacatgagagacaattggcggagcgagctgtacaagtacaaggtggtggaaatcaagcccctgggaatcgcccctaccggcgccaagagaagagtggtggaacgcgagaagcgggccgtgggaatcggagccgtgttcctgggatttctgggagccgccggaagcacaatgggcgctgccagcatcaccctgacagtgcaggctagacagctgctgagcggcatcgtgcagcagcagagcaacctgctgaaggccatcgaggcccagcagcatctgctgcagctgaccgtgtgggggatcaagcagctgcagaccagagtgctggccattgagagatacctgaaggaccagcagctgctgggcctgtggggctgttctgccaagctgatctgtaccaccgccgtgccttggaacagctcctggtccaacaagagcgaaaccgagatctggaacaatatgacatggatgcagtgggaccgcgagatcaacaattacaccaacaccatctaccggctgctggaagagagccagaaccagcaggaaaagaacgagaacgacctgctggccctggacaagtggaactccctgtgggattggttcggcatcagcaactggctgtggtacatccgcagccggatcgagggcagaggcagcggaggctatattcccgaggcccccagagatggccaggcctacgtgcggaaagatggcgagtgggtgctgctgagtaccttcctgggccaccatcaccaccaccac

SEQ ID NO: 28 - DNA, 2151 bp, Artificial Sequence
  Synthetic construct
atgagagtgcggggcatccagcggaattgccagcacctgtggcgctggggcacactgatcctgggcatgctgatgatctgcagcgccgtgggcaacctgtgggtcaccgtgtactatggcgtgcccgtgtggcgggaagccaagaccacactgttctgtgccagcgacgccaaggcctacgaccgcgaggtgcacaatgtgtgggccacccatgcctgcgtgcccaccgatcccaacccccaggaaatcgtgctggaaaacgtgaccgagaacttcaacatgtggaagaacgacatggtggaccagatgcacgaggacatcatcagcctgtgggaccagagcctgaagccctgcgtgaagctgacccctctgtgcgtgaccctgaactgcaccgccttcaacagcagcagccacaccaacagctctatcgccatgcaggaaatgaagaactgcagcttcaacgccaccaccgagatccgggaccggaagaaagagatgtacgccctgttctacaagctggacatcgtgcccatcaacaagaacggccggcagtaccggctgatcaactgcaacaccagcaccctgacccaggcctgccccaaggtgtccttcgaccccatccccatccactactgtacccctgccggcttcgccatcctgaagtgcaacaacaagaccttcaacggcaccggcccctgcaccaacgtgtccaccgtgcagtgtacccacggcatcaagcccgtggtgtccacccagctgctgctgaatggcagcctggccgaggaagatatcatcatcagaagcgagaacctgagcaacaacgccaagacaatcatcgtgcacctgaacgagagcgtggaaatcacctgtatccggcccagcaacaacaccagaaagagcgtgcggatcggccctggccagaccttctacgccaacaacgacatcatcggcaacatccggaaggcctactgcgagatcaacgagacaaagtggaacaacacactgcataatgtgtccaagaaactggtggaacacttccctaacaagaccaccatcagattcgaccggcactctggcggcgacctggaaattaccacccacagcttcaattgtggcggcgagttcttctactgcaatacctccggcctgttcaacatcagctacaacagcaactacacctacaacgacaccaagcacaacgggaccaaagtgatcaccctgccctgccggatcaagcagatcattaacatgtggcaggaagtgggcagggctatgtatgcccctcctatcgccggcaacattacctgcacctccaacatcaccggcctgctgctgaccagagatggcggcaacaactccaccgagacagagacattcagacccggcggaggcgacatgagagacaactggcggagcgagctgtacaagtacaaggtggtggaaatcaagcccctgggaatcgcccctaccggcgccaagagaagagtggtggaacgcgagaagcgggccgtgggaatcggagccgtgttcctgggatttctgggagccgccggaagcacaatgggcgctgccagcatcaccctgacagtgcaggctagacagctgctgagcggcatcgtgcagcagcagagcaacctgctgaaggccatcgaggcccagcagcatctgctgcagctgaccgtgtggggaatcaagcagctgcagacacgggtgctggccattgagagatacctgaaggaccagcagctgctgggcctgtggggctgttctgccaagctgatctgtaccaccgccgtgccctggaacagctcctggtccaacaagagcgaaaccgagatctggaacaatatgacctggatgcagtgggaccgggaaatcaacaattacaccaacaccatctaccggctgctggaagagagccagaaccagcaggaaaagaacgagaacgacctgctggccctggacaagtggaactccctgtgggattggttcggcatcagcaactggctgtggtacatccgcagccggatcgagggcagaggcagcggaggctatattcccgaggcccctagagatggccaggcctacgtgcggaaagacggcgaatgggtgctgctgtccaccttcctgggccaccatcaccaccaccac

SEQ ID NO: 29 - protein, 6 aa, Artificial Sequence
  Synthetic construct
HHHHHH

SEQ ID NO: 30 - protein, 711 aa, Artificial Sequence
  Synthetic construct
MRVRGIQRNCQHLWRWGTLILGMLMICSAVGNLWVTVYYGVPVWREAKTTLFCASDAKAYDREVHNVWATHACVPTDPNPQEIVLENVTENFNMWKNDMVDQMHEDIISLWDQSLKPCVKLTPLCVTLECTAFNSSSHTNSSIAMQEMKNCSFNMTTELRDKKKKVSALFYKLDIVPLNKNGRQYRLINCNTSTLTQACPKVSFDPIPIHYCTPAGYAILKCNNKTFNGTGPCNNVSTVQCTHGIKPVVSTQLLLNGSLAEEDIIIRSENLTNNAKTIIVHLNESVEIVCIRPNNNTRKSIRIGPGQTFYANNDIIGDIRQAHCNISKEKWNNTLHRVWKKLVEHFPNKTTIRFDRHSGGDLEITTHSFNCGGEFFYCNTSGLFNITYNSNYTYNDTKHNGTKVITLPCRIKQIINMWQEVGRAMYAPPIAGNITCTSNITGLLLTRDGGNNSTETETFRPGGGDMRDNWRSELYKYKVVEIKPLGIAPTGAKRRVVEREKRAVGIGAVFLGFLGAAGSTMGAASITLTVQARQLLSGIVQQQSNLLKAIEAQQHLLQLTVWGIKQLQTRVLAIERYLKDQQLLGLWGCSAKLICTTAVPWNSSWSNKSETEIWNNMTWMQWDREISNYTNTIYRLLEESQNQQEKNENDLLALDKWNSLWDWFGISNWLWYIRSRIEGRGSGGYIPEAPRDGQAYVRKDGEWVLLSTFLG

SEQ ID NO: 31 - protein, 711 aa, Artificial Sequence
  Synthetic construct
MRVRGIQRNCQHLWRWGTLILGMLMICSAVGNLWVTVYYGVPVWREAETTLFCASDAKAYDREVHNVWATHACVPTDPNPQEIVLENVTENFNMWKNDMVDQMHEDIISLWDQSLKPCVKLTPLCVTLDCKAFNSSSHTNSSIAMQEMKNCTFNITTSVKGKRQQEHALFYKLDIVPLNKNGRQYRLINCNTSTLTQACPKVSFDPIPIHYCTPAGYAILKCNNKTFNGTGPCNNVSTVQCTHGIKPVVSTQLLLNGSLAEEDIIIRSENLTNNAKTIIVHLNESVEIVCVRPNNNTRKSIRIGPGQTFYANNEIIGDIRQAHCNISKEKWNNTLHRVWKKLVEHFPNKTTIRFDRHSGGDLEITTHSFNCGGEFFYCNTSGLFNITYNSNYTYNDTKHNGTKVITLPCRIKQIINMWQEVGRAMYAPPIAGNITCTSNITGLLLTRDGGNNSTETETFRPGGGDMRDNWRSELYKYKVVEIKPLGIAPTGAKRRVVEREKRAVGIGAVFLGFLGAAGSTMGAASITLTVQARQLLSGIVQQQSNLLKAIEAQQHLLQLTVWGIKQLQTRVLAIERYLKDQQLLGLWGCSAKLICTTAVPWNSSWSNKSETEIWNNMTWMQWDREISNYTNTIYRLLEESQNQQEKNENDLLALDKWNSLWDWFGISNWLWYIRSRIEGRGSGGYIPEAPRDGQAYVRKDGEWVLLSTFLG

SEQ ID NO: 32 - protein, 725 aa, Artificial Sequence
  Synthetic construct
MDAMKRGLCCVLLLCGAVFVSPSASVGNLWVTVYYGVPVWREAKTTLFCASDAKAYDREVHNVWATHACVPTDPNPQEIVLENVTENFNMWKNDMVDQMHEDIISLWDQSLKPCVKLTPLCVTLNCTNVTSSAANVTSNVTNDANNASNANGRNVINEDMQNCSFNATTEIRDRKKEMYALFYKLDIVPLDGEKSDNRYRLINCNTSTLTQACPKVSFDPIPIHYCTPAGFAILKCNNKTFNGTGPCNNVSTVQCTHGIKPVVSTQLLLNGSLAEEDIIIRSENLTNNAKTIIVHLNESVEIVCTRPNNNTRKSIRIGPGQTFYANNDIIGDIRQAHCNISEEKWNNTLHRVWKKLVEHFPNKTTIRFDRHSGGDLEITTHSFNCGGEFFYCNTSGLFNITYNSNYTYNDTKHNGTKVITLPCRIKQIINMWQEVGRAMYAPPIAGNITCTSNITGLLLTRDGGNNSTETETFRPGGGDMRDNWRSELYKYKVVEIKPLGIAPTGAKSSVVERAKSAVGIGAVFLGFLGAAGSTMGAASITLTVQARQLLSGIVQQQSNLLKAIEAQQHLLQLTVWGIKQLQTRVLAIERYLKDQQLLGLWGCSAKLICTTAVPWNSSWSNKSETEIWNNMTWMQWDREINNYTNTIYRLLEESQNQQEKNENDLLALDKWNSLWDWFGISNWLWYIRSRIEGRGSGGYIPEAPRDGQAYVRKDGEWVLLSTFLG

SEQ ID NO: 33 - protein, 40 aa, Artificial Sequence
  Synthetic construct
CSFNMTTELRDKKKKVSALFYKLDIVPLNKNGRQYRLINC

SEQ ID NO: 34 - protein, 40 aa, Artificial Sequence
  Synthetic construct
CTFNITTSVKGKRQQEHALFYKLDIVPLNKNGRQYRLINC

SEQ ID NO: 35 - protein, 35 aa, Artificial Sequence
  Synthetic construct
CTRPGNNTRKSIRIGPGQTFYANNDIIGDIRQAHC

SEQ ID NO: 36 - protein, 35 aa, Artificial Sequence
  Synthetic construct
CIRPSNNTRKSVRIGPGQTFYANNDIIGNIRKAYC

SEQ ID NO: 37 - DNA, 118 bp, Artificial Sequence
  Synthetic construct
cgagctgcgggacaagaaaaagaaggtgtccgccctgttctacaagctggacatcgtgcccctgaacaagaacggccggcagtaccggctgatcaactgcaacaccagcaccctgacc

SEQ ID NO: 38 - DNA, 118 bp, Artificial Sequence
  Synthetic construct
cagcgtgaagggcaagcggcagcaggaacacgccctgttctacaagctggacatcgtgcccctgaacaagaacggccggcagtaccggctgatcaactgcaacaccagcaccctgacc

SEQ ID NO: 39 - DNA, 106 bp, Artificial Sequence
  Synthetic construct
caccagaaagagcatccggatcggccctggccagaccttctacgccaacaacgacatcatcggcgacatccggcaggcccactgcaacatctctgaggccaagtgg

SEQ ID NO: 40 - DNA, 106 bp, Human immunodeficiency virus type 1
caccagaaagagcgtgcggatcggccctggccagaccttctacgccaacaacgacatcatcggcaacatccggaaggcctactgcgagatcaacgagacaaagtgg

SEQ ID NO: 41 - protein, 714 aa, Artificial Sequence
  Synthetic construct (C97ZA012 gp140Fd)
MRVRGIQRNCQHLWRWGTLILGMLMICSAAENLWVGNMWVTVYYGVPVWTDAKTTLFCASDTKAYDREVHNVWATHACVPTDPNPQEIVLENVTENFNMWKNDMVDQMHEDIISLWDQSLKPCVKLTPLCVTLHCTNATFKNNVTNDMNKEIRNCSFNTTTEIRDKKQQGYALFYRPDIVLLKENRNNSNNSEYILINCNASTITQACPKVNFDPIPIHYCAPAGYAILKNNKTFSGKGPCNNVSTVQCTHGIKPVVSTQLLLNGSLAEKEIIIRSENLTDNVKTIIVHLNKSVEIVCTRPNNNTRKSMRIGPGQTFYATGDIIGDIRQAYCNISGSKWNETLKRVKEKLQENYNNNKTIKFAPSSGGDLEITTHSFNCRGEFFYCNTTRLFNNNATEDETITLPCRIKQIINMWQGVGRAMYAPPIAGNITCKSNITGLLLVRDGGEDNKTEEIFRPGGGNMKDNWRSELYKYKVIELKPLGIAPTGAKRRVVEREKRAVGIGAVFLGFLGAAGSTMGAASLTLTVQARQLLSSIVQQQSNLLRAIEAQQHMLQLTVWGIKQLQTRVLAIERYLKDQQLLGIWGCSGKLICTTNVPWNSSWSNKSQTDIWNNMTWMEWDREISNYTDTIYRLLEDSQTQQEKNEKDLLALDSWKNLWSWFDISNWLWYIKSRIEGRGSGGYIPEAPRDGQAYVRKDGEWVLLSTFLGHHHHHH

SEQ ID NO: 42 - protein, 723 aa, Artificial Sequence
  Synthetic construct (92UG037.8 gp140Fd)
MRVRGIQRNCQHLWRWGTLILGMLMICSAAENLWVTVYYGVPVWKDAETTLFCASDAKAYDTEVHNVWATHACVPTDPNPQEIYMENVTEEFNMWKNNMVEQMHTDIISLWDQSLKPCVQLTPLCVTLDCSYNITNNITNSITNSSVNMREEIKNCSFNMTTELRDKNRKVYSLFYKLDVVQINNGNNSSNLYRLINCNTSALTQACPKVTFEPIPIRYCAPAGYAILKCNDKEFNGTGLCKNVSTVQCTHGIRPVVSTQLLLNGSLAEGKVMIRSENITNNVKNIIVQLNETVTINCTRPNNNTRKSVRIGPGQTFYATGDIIGDIRQAHCNVSGSQWNRALHQVVGQLREYWNTTIIFKNSSGGDLEITTHSFNCGGEFFYCNTSGLFNSNWTHNDTASMKPNDTITLPCRIKQIINMWQRVGQAIYAPPIQGVIRCESNITGLILTRDGGGNINESQIFRPGGGDMRDNWRSELYKYKVVRIEPLGVAPTKAKRRVVEREKRAVVELGAVFIGFLGTAGSTMGAASITLTVQVRKLLSGIVQQQSNLLRAIEAQQHLLKLTVWGIKQLQARVLAVERYLRDQQLLGIWGCSGKLICTTNVPWNSSWSNKSEREIWENMTWLQWDKEISNYTHIIYELIEESQKQQEKNEQELLELDKWANLWNWFDISNWLWYIKEFSRIEGRGSGGYIPEAPRDGQAYVRKDGEWVLLSTFLGHHHHHH

SEQ ID NO: 43 - protein, 719 aa, Artificial Sequence
  Synthetic construct (Mosaic 3.1 gp140Fd)
MRVTGIRKNYQHLWRWGTMLLGILMICSAAGKLWVTVYYGVPVWKEATTTLFCASDAKAYDTEVHNVWATHACVPTDPNPQEVVLENVTENFNMWKNNMVEQMHEDIISLWDQSLKPCVKLTPLCVTLNCTDDVRNVTNNATNTNSSWGEPMEKGEIKNCSFNITTSIRNKVQKQYALFYKLDVVPIDNDSNNTNYRLISCNTSVITQACPKVSFEPIPIHYCAPAGFAILKCNDKKFNGTGPCTNVSTVQCTHGIRPVVSTQLLLNGSLAEEEVVIRSENFTNNAKTIMVQLNVSVEINCTRPNNNTRKSIHIGPGRAFYTAGDIIGDIRQAHCNISRANWNNTLRQIVEKLGKQFGNNKTIVFNHSSGGDPEIVMHSFNCGGEFFYCNSTKLFNSTWTWNNSTWNNTKRSNDTEEHITLPCRIKQIINMWQEVGKAMYAPPIRGQIRCSSNITGLLLTRDGGNDTSGTEIFRPGGGDMRDNWRSELYKYKVVKIEPLGVAPTKAKRRVVQSEKSAVGIGAVFLGFLGAAGSTMGAASMTLTVQARLLLSGIVQQQNNLLRAIEAQQHLLQLTVWGIKQLQARVLAVERYLKDQQLLGIWGCSGKLICTTTVPWNASWSNKSLDKIWNNMTWMEWEREINNYTSLIYTLIEESQNQQEKNEQELLELDKWASLWNWFDISNWLWGYIPEAPRDGQAYVRKDGEWVLLSTFLGHHHHHH

SEQ ID NO: 44 - protein, 714 aa, Artificial Sequence
  Synthetic construct (405C gp140Fd)
MRVRGIQRNCQHLWRWGTLILGMLMICSAVGNMWVTVYYGVPVWTEAKATLFCASDAKAYEKEVHNVWATHACVPTDPNPQEIILENVTENFNMWKNDMVDQMHEDIISIWDQSLKPCVKLTPLCVTLTCKNITNNVTNIFNSSEGINMKEEIKNCSFNTTTEIRDKEKKEYALFYKPDIVQLGERNSSRYILINCNSSTITQACPKVTFDPIPIHYCAPAGYAILKCNNKTFNGTGPCSNISTVQCTHGIKPVVSTQLLLNGSLSEGEIMIRSENLTDNTKTIIVHLNESVEIVCIRPGNNTRKGIRIGPGQVFYATGDIIGDIRQAYCNISGKWNTTLEKVKKKLKEHFPNKTINFNSSSGGDLEITTHSFNCRGEFFYCNTTKLFTNTTTNTTILIPCRIKQFVNMWQEVGRAMYAPPIAGNITCNSSITGLLLVRDGGISNDTNNTTETFRPGGGNMKDNWRSELYSYKVVELKPLGVAPTGAKRRVVEMERSKRAVGIGAALLGFLGAAGSTMGAASMALTVQARQLLSGIVQQQSNLLRAIEAQQHMLQLTVWGIKQLQTRVLAIERYLKDQQLLGLWGCSGKIICTTNVPWNSSWSNKSKEDIWDNMTWMQWDREVSNYTETIYRLLEESQTQQEKNEKELLELSKWDSLWSWFNITNWLWYTKSRIEGRGSGGYIPEAPRDGQAYVRKDGEWVLLSTFLGHHHHHH

SEQ ID NO: 45 - protein, 701 aa, Artificial Sequence
  Synthetic construct (PVO.4 gp140Fd)
MRVTGIRKNYQHSWRWGMMLLGMLMICSAEEKLWVTVYYGVPVWKEATTTLFCASDAKAYNTEVHNVWATHACVPTDPNPQEVGLENVTENFNMWKNNMVEQMHEDIISLWDQSLKPCVKLTPLCVTLNCSDLRNATNTTNPTVSSRVIKKEMMGEVKNCSFNVTTDIRDRMQKVYALFYRPDVVPIQDHTIENNNTIENNTTYRLISCNTSVITQACPKISFEPIPIHYCTPAGFAILKCNDKKFNGSGPCTNVSTVQCTHGIRPVVSTQLLLNGSRAEEEVIIRSENFTNNAKTIIVQLNKTVEINCTRPNNNTRKSISIGPGRAFYATGDIIGDIRQAHCNLSRAEWNTLKYISTKLREQFGNKTIIFNGSSGGDPEIVTHSFNCGGEFFYCNTTKLFNSTWDANGNCTGCDESDGNNTITLPCRIKQIVNMWQEVGKAMYAPPIKGLIKCTSNITGLLLTRDGGANNTNETFRPGGGDMRDNWRSELYKYKVVQIEPLGIAPTRARRRVVQREKRAVGTLGAMFLGFLGAAGSTMGAASVTLTVQARQLLSGIVQQQNNLLKAIEAQQHMLQLTVWGIKQLQARVLAIERYLKDQQLLGIWGCSGKLICTTAVPWNTSWSNKSFNKIWDNMTWMEWEREIDNYTGLIYNLLEESQNQQEKNEQDLLALDKWESLWNWFSITKWLWYIKGSGHHHHHH

SEQ ID NO: 46 - protein, 856 aa, Artificial Sequence
  Synthetic construct (HXB2)
MRVKEKYQHLWRWGWRWGTMLLGMLMICSATEKLWVTVYYGVPVWKEATTTLFCASDAKAYDTEVHNVWATHACVPTDPNPQEVVLVNVTENFNMWKNDMVEQMHEDIISLWDQSLKPCVKLTPLCVSLKCTDLKNDTNTNSSSGRMIMEKGEIKNCSFNISTSIRGKVQKEYAFFYKLDIIPIDNDTTSYKLTSCNTSVITQACPKVSFEPIPIHYCAPAGFAILKCNNKTFNGTGPCTNVSTVQCTHGIRPVVSTQLLLNGSLAEEEVVIRSVNFTDNAKTIIVQLNTSVEINCTRPNNNTRKRIRIQRGPGRAFVTIGKIGNMRQAHCNISRAKWNNTLKQIASKLREQFGNNKTIIFKQSSGGDPEIVTHSFNCGGEFFYCNSTQLFNSTWFNSTWSTEGSNNTEGSDTITLPCRIKQIINMWQKVGKAMYAPPISGQIRCSSNITGLLLTRDGGNSNNESEIFRPGGGDMRDNWRSELYKYKVVKIEPLGVAPTKAKRRVVQREKRAVGIGALFLGFLGAAGSTMGAASMTLTVQARQLLSGIVQQQNNLLRAIEAQQHLLQLTVWGIKQLQARILAVERYLKDQQLLGIWGCSGKLICTTAVPWNASWSNKSLEQIWNHTTWMEWDREINNYTSLIHSLIEESQNQQEKNEQELLELDKWASLWNWFNITNWLWYIKLFIMIVGGLVGLRIVFAVLSIVNRVRQGYSPLSFQTHLPTPRGPDRPEGIEEEGGERDRDRSIRLVNGSLALIWDDLRSLCLFSYHRLRDLLLIVTRIVELLGRRGWEALKYWWNLLQYWSQELKNSAVSLLNATAIAVAEGTDRVIEVVQGACRAIRHIPRRIRQGLERILL